European Patent Application EP 4 458 369 A1, published November 6, 2024. Title: 质子泵调控剂在制备试剂中的用途. Applicant: 上海魁特迪生物科技有限公司. The sequence listing filed with the application follows.

SEQUENCE LISTING (18 sequences)

SEQ ID NO: 1 - protein, 19 aa, synthetic construct
  REGION 1..19: note = QD202
YGRKKRRQRRRSPVDVVCS

SEQ ID NO: 2 - protein, 18 aa, synthetic construct
  REGION 1..18: note = QD202 N -1
YGRKKRRQRRRPVDVVCS

SEQ ID NO: 3 - protein, 18 aa, synthetic construct
  REGION 1..18: note = QD202 C -1
YGRKKRRQRRRSPVDVVC

SEQ ID NO: 4 - protein, 17 aa, synthetic construct
  REGION 1..17: note = QD202 C -2
YGRKKRRQRRRSPVDVV

SEQ ID NO: 5 - protein, 19 aa, synthetic construct
  REGION 1..19: note = QD202
  SITE 19: note = misc_feature - Xaa = Ser
YGRKKRRQRRRSPVDVVCX

SEQ ID NO: 6 - protein, 775 aa, synthetic construct
  REGION 1..775: note = ATP6V1B2-mCherry
MALRAMRGIVNGAAPELPVPTGGPMAGAREQALAVSRNYLSQPRLTYKTVSGVNGPLVILDHVKFPRYAEIVHLTLPDGTKRSGQVLEVSGSKAVVQVFEGTSGIDAKKTSCEFTGDILRTPVSEDMLGRVFNGSGKPIDRGPVVLAEDFLDIMGQPINPQCRIYPEEMIQTGISAIDGMNSIARGQKIPIFSAAGLPHNEIAAQICRQAGLVKKSKDVVDYSEENFAIVFAAMGVNMETARFFKSDFEENGSMDNVCLFLNLANDPTIERIITPRLALTTAEFLAYQCEKHVLVILTDMSSYAEALREVSAAREEVPGRRGFPGYMYTDLATIYERAGRVEGRNGSITQIPILTMPNDDITHPIPDLTGYITEGQIYVDRQLHNRQIYPPINVLPSLSRLMKSAIGEGMTRKDHADVSNQLYACYAIGKDVQAMKAVVGEEALTSDDLLYLEFLQKFEKNFITQGPYENRTVYETLDIGWQLLRIFPKEMLKRIPQSTLSEFYPRDSAKHEQKLISEEDLATNFSLLKQAGDVEENPGPVSKGEEDNMAIIKEFMRFKVHMEGSVNGHEFEIEGEGEGRPYEGTQTAKLKVTKGGPLPFAWDILSPQFMYGSKAYVKHPADIPDYLKLSFPEGFKWERVMNFEDGGVVTVTQDSSLQDGEFIYKVKLRGTNFPSDGPVMQKKTMGWEASSERMYPEDGALKGEIKQRLKLKDGGHYDAEVKTTYKAKKPVQLPGAYNVNIKLDITSHNEDYTIVEQYERAEGRHSTGGMDELYK

SEQ ID NO: 7 - protein, 19 aa, synthetic construct
  REGION 1..19: note = QD201
YGRKKRRQRRRVCDSSVVP

SEQ ID NO: 8 - protein, 512 aa, Mus musculus
  SITE 512: note = misc_feature - Xaa =
MALRAMRGIVNGAAPELPVPTGGPMAGAREQALAVSRNYLSQPRLTYKTVSGVNGPLVILDHVKFPRYAEIVHLTLPDGTKRSGQVLEVSGSKAVVQVFEGTSGIDAKKTSCEFTGDILRTPVSEDMLGRVFNGSGKPIDRGPVVLAEDFLDIMGQPINPQCRIYPEEMIQTGISAIDGMNSIARGQKIPIFSAAGLPHNEIAAQICRQAGLVKKSKDVVDYSEENFAIVFAAMGVNMETARFFKSDFEENGSMDNVCLFLNLANDPTIERIITPRLALTTAEFLAYQCEKHVLVILTDMSSYAEALREVSAAREEVPGRRGFPGYMYTDLATIYERAGRVEGRNGSITQIPILTMPNDDITHPIPDLTGYITEGQIYVDRQLHNRQIYPPINVLPSLSRLMKSAIGEGMTRKDHADVSNQLYACYAIGKDVQAMKAVVGEEALTSDDLLYLEFLQKFEKNFITQGPYENRTVYETLDIGWQLLRIFPKEMLKRIPQSTLSEFYPRDSAKHX

SEQ ID NO: 9 - DNA, 1536 bp, Mus musculus
  source 1..1536: mol_type = genomic DNA
atggcgttgcgagcgatgcggggaatcgtgaacggggccgcacccgaactgcccgtgcccaccggtgggccgatggccggagctcgggagcaggcgctggcggtgagccggaactacctatcccagcctcgtctcacctacaagactgtctctggggtgaatggtccactagtgatcctagatcatgtgaagtttcccagatacgctgagattgtccacttgacattaccagatggcacaaagagaagtgggcaagtcctagaagttagtggctccaaagcagtggttcaggtatttgaagggacatctggtatagacgccaagaaaacatcctgtgagtttactggagatattctccgaacaccagtgtctgaggatatgcttggtcgagtattcaacggatcaggaaaacccattgaccgaggccctgtggtgctggctgaagacttccttgacatcatgggtcagccaatcaaccctcagtgtcggatctatccagaagagatgattcagacgggcatttccgccatcgatggcatgaacagtattgctaggggacagaaaatccccatcttttctgctgctggattaccacacaacgagattgcagctcagatctgtcgccaggctggtttggtaaagaaatccaaagatgtagtggactatagtgaagaaaattttgccattgtgtttgctgctatgggagtaaacatggaaacagcccggttctttaaatctgactttgaagaaaatggctcaatggacaatgtctgcctttttttgaatctggctaatgacccaaccattgagcggatcatcactcctcgcctggctctgaccacggccgagtttctggcatatcagtgtgagaagcacgtgctggtgatcctgacggacatgagctcctacgctgaagcgctgcgagaggtttcagctgccagggaagaggtccctggtcggcgaggcttcccaggctacatgtataccgacttagccacaatctatgaacgtgccggtcgagtggaaggtagaaacggctctattacccaaatccctattctcaccatgcccaatgacgatatcactcatcccatccctgacttgactgggtacattactgagggccagatctatgtggacagacagctgcacaacagacagatttaccctcctattaatgtgctgccctcactctctcggttaatgaagtcagctatcggagaaggaatgaccagaaaggatcacgctgatgtgtctaaccagttgtatgcgtgctatgccatcggtaaggacgtgcaagccatgaaagccgtggtgggagaggaagccctgacctcagatgatctcctttacctggaatttctgcagaagtttgagaagaacttcattactcagggtccctatgaaaaccgaactgtttatgagactttggacattggctggcagttgcttcgaatcttccccaaagaaatgctgaagagaatccctcagagcaccctgagcgaattttaccctcgagactctgcaaaacactag

SEQ ID NO: 10 - protein, 286 aa, synthetic construct
  REGION 1..286: note = ATP6V1B2 1-286aa
MALRAMRGIVNGAAPELPVPTGGPMAGAREQALAVSRNYLSQPRLTYKTVSGVNGPLVILDHVKFPRYAEIVHLTLPDGTKRSGQVLEVSGSKAVVQVFEGTSGIDAKKTSCEFTGDILRTPVSEDMLGRVFNGSGKPIDRGPVVLAEDFLDIMGQPINPQCRIYPEEMIQTGISAIDGMNSIARGQKIPIFSAAGLPHNEIAAQICRQAGLVKKSKDVVDYSEENFAIVFAAMGVNMETARFFKSDFEENGSMDNVCLFLNLANDPTIERIITPRLALTTAEFLA

SEQ ID NO: 11 - protein, 172 aa, synthetic construct
  REGION 1..172: note = ATP6V1B2 1-172aa
MALRAMRGIVNGAAPELPVPTGGPMAGAREQALAVSRNYLSQPRLTYKTVSGVNGPLVILDHVKFPRYAEIVHLTLPDGTKRSGQVLEVSGSKAVVQVFEGTSGIDAKKTSCEFTGDILRTPVSEDMLGRVFNGSGKPIDRGPVVLAEDFLDIMGQPINPQCRIYPEEMIQT

SEQ ID NO: 12 - protein, 551 aa, synthetic construct
  REGION 1..551: note = ATP6V1B2 Myc
  SITE 551: note = misc_feature - Xaa =
MALRAMRGIVNGAAPELPVPTGGPMAGAREQALAVSRNYLSQPRLTYKTVSGVNGPLVILDHVKFPRYAEIVHLTLPDGTKRSGQVLEVSGSKAVVQVFEGTSGIDAKKTSCEFTGDILRTPVSEDMLGRVFNGSGKPIDRGPVVLAEDFLDIMGQPINPQCRIYPEEMIQTGISAIDGMNSIARGQKIPIFSAAGLPHNEIAAQICRQAGLVKKSKDVVDYSEENFAIVFAAMGVNMETARFFKSDFEENGSMDNVCLFLNLANDPTIERIITPRLALTTAEFLAYQCEKHVLVILTDMSSYAEALREVSAAREEVPGRRGFPGYMYTDLATIYERAGRVEGRNGSITQIPILTMPNDDITHPIPDLTGYITEGQIYVDRQLHNRQIYPPINVLPSLSRLMKSAIGEGMTRKDHADVSNQLYACYAIGKDVQAMKAVVGEEALTSDDLLYLEFLQKFEKNFITQGPYENRTVYETLDIGWQLLRIFPKEMLKRIPQSTLSEFYPRDSAKHEFCRYPAQWRPLESRGPFEQKLISEEDLNMHTGHHHHHHX

SEQ ID NO: 13 - protein, 326 aa, synthetic construct
  REGION 1..326: note = ATP6V1B2 1-286aa Myc
  SITE 326: note = misc_feature - Xaa =
MALRAMRGIVNGAAPELPVPTGGPMAGAREQALAVSRNYLSQPRLTYKTVSGVNGPLVILDHVKFPRYAEIVHLTLPDGTKRSGQVLEVSGSKAVVQVFEGTSGIDAKKTSCEFTGDILRTPVSEDMLGRVFNGSGKPIDRGPVVLAEDFLDIMGQPINPQCRIYPEEMIQTGISAIDGMNSIARGQKIPIFSAAGLPHNEIAAQICRQAGLVKKSKDVVDYSEENFAIVFAAMGVNMETARFFKSDFEENGSMDNVCLFLNLANDPTIERIITPRLALTTAEFLAEFCRYPAQWRPLESRGPFEQKLISEEDLNMHTGHHHHHHX

SEQ ID NO: 14 - protein, 212 aa, synthetic construct
  REGION 1..212: note = ATP6V1B2 1-172aa Myc
  SITE 212: note = misc_feature - Xaa =
MALRAMRGIVNGAAPELPVPTGGPMAGAREQALAVSRNYLSQPRLTYKTVSGVNGPLVILDHVKFPRYAEIVHLTLPDGTKRSGQVLEVSGSKAVVQVFEGTSGIDAKKTSCEFTGDILRTPVSEDMLGRVFNGSGKPIDRGPVVLAEDFLDIMGQPINPQCRIYPEEMIQTEFCRYPAQWRPLESRGPFEQKLISEEDLNMHTGHHHHHHX

SEQ ID NO: 15 - protein, 270 aa, synthetic construct
  REGION 1..270: note = QD202-EGFP
  SITE 270: note = misc_feature - Xaa =
MYGRKKRRQRRRSPVDVVCSGTAGPGSIATMVSKGEELFTGVVPILVELDGDVNGHKFSVSGEGEGDATYGKLTLKFICTTGKLPVPWPTLVTTLTYGVQCFSRYPDHMKQHDFFKSAMPEGYVQERTIFFKDDGNYKTRAEVKFEGDTLVNRIELKGIDFKEDGNILGHKLEYNYNSHNVYIMADKQKNGIKVNFKIRHNIEDGSVQLADHYQQNTPIGDGPVLLPDNHYLSTQSALSKDPNEKRDHMVLLEFVTAAGITLGMDELYKX

SEQ ID NO: 16 - protein, 512 aa, Homo sapiens
  SITE 512: note = misc_feature - Xaa =
MALRAMRGIVNGAAPELPVPTGGPAVGAREQALAVSRNYLSQPRLTYKTVSGVNGPLVILDHVKFPRYAEIVHLTLPDGTKRSGQVLEVSGSKAVVQVFEGTSGIDAKKTSCEFTGDILRTPVSEDMLGRVFNGSGKPIDRGPVVLAEDFLDIMGQPINPQCRIYPEEMIQTGISAIDGMNSIARGQKIPIFSAAGLPHNEIAAQICRQAGLVKKSKDVVDYSEENFAIVFAAMGVNMETARFFKSDFEENGSMDNVCLFLNLANDPTIERIITPRLALTTAEFLAYQCEKHVLVILTDMSSYAEALREVSAAREEVPGRRGFPGYMYTDLATIYERAGRVEGRNGSITQIPILTMPNDDITHPIPDLTGYITEGQIYVDRQLHNRQIYPPINVLPSLSRLMKSAIGEGMTRKDHADVSNQLYACYAIGKDVQAMKAVVGEEALTSDDLLYLEFLQKFERNFIAQGPYENRTVFETLDIGWQLLRIFPKEMLKRIPQSTLSEFYPRDSAKHX

SEQ ID NO: 17 - DNA, 1536 bp, Homo sapiens
  source 1..1536: mol_type = genomic DNA
atggcgctgcgggcgatgcgggggattgtcaacggggccgcacccgagctacccgtgcccaccggtgggccggcggtgggagctcgggagcaggcgctggcagtcagtcggaactacctctcccagcctcgcctcacatacaagacagtatctggagtcaatggtccactagtgatcttagatcatgttaagtttcccaggtatgctgaaattgtccatttgaccttaccggatggcacaaagagaagtgggcaagttctggaagttagtggttccaaggcagtagttcaggtatttgaagggacttcaggtatagatgctaagaaaacgtcctgtgagtttactggggatattctccgaacaccggtgtctgaggatatgcttggtcgggtattcaatggatcgggaaaacccattgacagaggtcctgttgtactggccgaagacttccttgatatcatgggtcagccaatcaaccctcaatgtcgaatctacccagaggaaatgattcagactggcatttcggccatcgatgggatgaacagtattgctagggggcagaaaattcctatcttctctgctgctgggctaccacacaatgagattgcagctcagatctgtcgccaggctggtttggtaaagaaatccaaagatgtagtagactacagtgaggaaaattttgcaattgtatttgctgctatgggtgtaaacatggaaactgcccggttcttcaaatctgactttgaagaaaatggctcaatggacaatgtctgcctctttttgaacttggctaatgacccaaccattgagcgaattatcactcctcgcctggctctaaccacagctgaatttctggcgtaccaatgtgagaaacatgtattggttattctaacagacatgagttcttatgctgaagcacttcgagaggtttcagcagccagggaagaggtacctggtcgacgaggttttccaggttacatgtatacagatttagccacgatatatgaacgcgctgggcgagtggaagggagaaacggctcgattactcaaatccctattctaaccatgcctaatgatgatatcactcaccccatcccagacttgactggctacattacagaggggcagatctatgtggacagacagctgcacaacagacagatttatccacctatcaatgtgctgccctcactatcacggttaatgaagtctgctattggagaagggatgaccaggaaggatcatgccgatgtatctaaccagctatatgcgtgctatgctattggaaaggatgtgcaagccatgaaagctgtcgttggagaagaagcccttacctcagatgatcttctctacttggaatttctgcagaagtttgagaggaacttcattgctcagggtccttacgaaaatcgcactgtctttgagactttggacattggctggcagctactccgaatcttccccaaagaaatgctgaagagaatccctcagagcaccctcagcgaattttaccctcgagactctgcaaagcattag

SEQ ID NO: 18 - protein, 38 aa, synthetic construct
  REGION 1..38: note = QD202
YGRKKRRQRRRSPVDVVCSSCVVDVPSRRRQRRKKRGY